European Patent Specification EP 4 185 693 B1, published February 11, 2026. Title: Combinatorial inhibition of transcription factors for treatment of heart failure. Applicant: Goethe Universitaet. The sequence listing filed with the application follows.

SEQUENCE LISTING (188 sequences)

SEQ ID NO: 1 - RNA, 19 nt, Artificial Sequence
  siRNA
gcaaguacacuacgaacaa

SEQ ID NO: 2 - RNA, 19 nt, Artificial Sequence
  siRNA
cgaaucugcacgcgguaca

SEQ ID NO: 3 - RNA, 19 nt, Artificial Sequence
  siRNA
aagacaagucauccggcua

SEQ ID NO: 4 - RNA, 19 nt, Artificial Sequence
  siRNA
gcucaaaccacuccaucga

SEQ ID NO: 5 - RNA, 19 nt, Artificial Sequence
  siRNA
gcacuuaccagcugacgua

SEQ ID NO: 6 - RNA, 19 nt, Artificial Sequence
  siRNA
ggagagggauuuagccgau

SEQ ID NO: 7 - RNA, 19 nt, Artificial Sequence
  siRNA
gcacacaucguuucgaaca

SEQ ID NO: 8 - RNA, 19 nt, Artificial Sequence
  siRNA
caaaacagcuccuccgauu

SEQ ID NO: 9 - RNA, 19 nt, Artificial Sequence
  siRNA
ugacaaagaaaacgaaaga

SEQ ID NO: 10 - RNA, 19 nt, Artificial Sequence
  siRNA
ccggaagaggcguguguau

SEQ ID NO: 11 - RNA, 19 nt, Artificial Sequence
  siRNA
ggauaggaucugaccugaa

SEQ ID NO: 12 - RNA, 19 nt, Artificial Sequence
  siRNA
gacgaguugauuaaagauu

SEQ ID NO: 13 - RNA, 19 nt, Artificial Sequence
  siRNA
gggcgaaugucguagccga

SEQ ID NO: 14 - RNA, 19 nt, Artificial Sequence
  siRNA
cgucacacaucccgucaga

SEQ ID NO: 15 - RNA, 19 nt, Artificial Sequence
  siRNA
cgaagaggagggcgacuua

SEQ ID NO: 16 - RNA, 19 nt, Artificial Sequence
  siRNA
caauaugaauagcgaccca

SEQ ID NO: 17 - RNA, 19 nt, Artificial Sequence
  siRNA
gcaucuaugacaucguaaa

SEQ ID NO: 18 - RNA, 19 nt, Artificial Sequence
  siRNA
agaagagcgaggccgcaaa

SEQ ID NO: 19 - RNA, 19 nt, Artificial Sequence
  siRNA
caacggagacaucgggaga

SEQ ID NO: 20 - RNA, 19 nt, Artificial Sequence
  siRNA
ggauaaauguauauacgug

SEQ ID NO: 21 - RNA, 19 nt, Artificial Sequence
  siRNA
aauaaguagcuguaacgua

SEQ ID NO: 22 - RNA, 19 nt, Artificial Sequence
  siRNA
gcaugguaacuuagccgaa

SEQ ID NO: 23 - RNA, 19 nt, Artificial Sequence
  siRNA
aaucuuguguacaucguaa

SEQ ID NO: 24 - RNA, 19 nt, Artificial Sequence
  siRNA
caucggaggaagucauuau

SEQ ID NO: 25 - RNA, 19 nt, Artificial Sequence
  siRNA
gugcagaaacgacgcaucu

SEQ ID NO: 26 - RNA, 19 nt, Artificial Sequence
  siRNA
ccauggaagaagaccgguu

SEQ ID NO: 27 - RNA, 19 nt, Artificial Sequence
  siRNA
gcuuaaagguuuuccgauc

SEQ ID NO: 28 - RNA, 19 nt, Artificial Sequence
  siRNA
acucagacauccagcgccu

SEQ ID NO: 29 - RNA, 19 nt, Artificial Sequence
  siRNA
agacagugauugcggucaa

SEQ ID NO: 30 - RNA, 19 nt, Artificial Sequence
  siRNA
gcauccagcucauccgcaa

SEQ ID NO: 31 - RNA, 19 nt, Artificial Sequence
  siRNA
ccuacuacacuucgcuuua

SEQ ID NO: 32 - RNA, 19 nt, Artificial Sequence
  siRNA
caagauuggaagugccgga

SEQ ID NO: 33 - RNA, 19 nt, Artificial Sequence
  siRNA
cauagcgacugcucgguuu

SEQ ID NO: 34 - RNA, 19 nt, Artificial Sequence
  siRNA
ucaauagagagccuacaaa

SEQ ID NO: 35 - RNA, 19 nt, Artificial Sequence
  siRNA
cuguuauaguugugaaagc

SEQ ID NO: 36 - RNA, 19 nt, Artificial Sequence
  siRNA
agaggaggaucuacgacau

SEQ ID NO: 37 - RNA, 19 nt, Artificial Sequence
  siRNA
ccgggagauugccgacaaa

SEQ ID NO: 38 - RNA, 19 nt, Artificial Sequence
  siRNA
gguauuggucugaucgaga

SEQ ID NO: 39 - RNA, 19 nt, Artificial Sequence
  siRNA
ggaaugucgcagaggacgu

SEQ ID NO: 40 - RNA, 19 nt, Artificial Sequence
  siRNA
acuccaagccggcacgaga

SEQ ID NO: 41 - RNA, 19 nt, Artificial Sequence
  siRNA
ugauaucaccaacgucuua

SEQ ID NO: 42 - RNA, 19 nt, Artificial Sequence
  siRNA
gaucuagaauugaaggaaa

SEQ ID NO: 43 - RNA, 19 nt, Artificial Sequence
  siRNA
gcaguugcuuuaaugguga

SEQ ID NO: 44 - RNA, 19 nt, Artificial Sequence
  siRNA
agacauucacugccauaua

SEQ ID NO: 45 - RNA, 19 nt, Artificial Sequence
  siRNA
acacagaucauccgaguuu

SEQ ID NO: 46 - RNA, 19 nt, Artificial Sequence
  siRNA
ccaaacaguaucaccgcau

SEQ ID NO: 47 - RNA, 19 nt, Artificial Sequence
  siRNA
ggacaaggccaaacuauca

SEQ ID NO: 48 - RNA, 19 nt, Artificial Sequence
  siRNA
uggaagaagagccguugua

SEQ ID NO: 49 - RNA, 19 nt, Artificial Sequence
  siRNA
gaggauaacaagcgucgua

SEQ ID NO: 50 - RNA, 19 nt, Artificial Sequence
  siRNA
ccggccaguugcaguauau

SEQ ID NO: 51 - RNA, 19 nt, Artificial Sequence
  siRNA
acgugugguugaagaaaua

SEQ ID NO: 52 - RNA, 19 nt, Artificial Sequence
  siRNA
gcuauguguccaaugcuau

SEQ ID NO: 53 - RNA, 19 nt, Artificial Sequence
  siRNA
caucuuaacacacgcuaaa

SEQ ID NO: 54 - RNA, 19 nt, Artificial Sequence
  siRNA
agggauaacucugcuauga

SEQ ID NO: 55 - RNA, 19 nt, Artificial Sequence
  siRNA
gggcgacacccucuacauu

SEQ ID NO: 56 - RNA, 19 nt, Artificial Sequence
  siRNA
gcgccgacccggguaauaa

SEQ ID NO: 57 - RNA, 19 nt, Artificial Sequence
  siRNA
ccucauagcccucggguac

SEQ ID NO: 58 - RNA, 19 nt, Artificial Sequence
  siRNA
gagaagugccucagcguag

SEQ ID NO: 59 - RNA, 19 nt, Artificial Sequence
  siRNA
gaauaguaacgccgacuca

SEQ ID NO: 60 - RNA, 19 nt, Artificial Sequence
  siRNA
ggcccauaaucuccgauau

SEQ ID NO: 61 - RNA, 19 nt, Artificial Sequence
  siRNA
gcacuaaggcucuagguac

SEQ ID NO: 62 - RNA, 19 nt, Artificial Sequence
  siRNA
cagcuagaguacaacgguu

SEQ ID NO: 63 - RNA, 19 nt, Artificial Sequence
  siRNA
cugcaaaccguaauccgua

SEQ ID NO: 64 - RNA, 19 nt, Artificial Sequence
  siRNA
ccaacauggcagucgguaa

SEQ ID NO: 65 - RNA, 19 nt, Artificial Sequence
  siRNA
ugagagaaaugcuuacaca

SEQ ID NO: 66 - RNA, 19 nt, Artificial Sequence
  siRNA
ggaaacgagugaaaggaua

SEQ ID NO: 67 - RNA, 19 nt, Artificial Sequence
  siRNA
uuacugaguugauggguua

SEQ ID NO: 68 - RNA, 19 nt, Artificial Sequence
  siRNA
cugauaacgugaacaaaua

SEQ ID NO: 69 - RNA, 19 nt, Artificial Sequence
  siRNA
cgagauaggcauacagcgu

SEQ ID NO: 70 - RNA, 19 nt, Artificial Sequence
  siRNA
ccuaccagacaucgaggaa

SEQ ID NO: 71 - RNA, 19 nt, Artificial Sequence
  siRNA
aggaagauggauuggcguu

SEQ ID NO: 72 - RNA, 19 nt, Artificial Sequence
  siRNA
aggaggaaccagagaucga

SEQ ID NO: 73 - RNA, 19 nt, Artificial Sequence
  siRNA
cgacuaaccguuggcgaga

SEQ ID NO: 74 - RNA, 19 nt, Artificial Sequence
  siRNA
ucuaauagccuaaacgaug

SEQ ID NO: 75 - RNA, 19 nt, Artificial Sequence
  siRNA
ccgaggaguucaacgaucu

SEQ ID NO: 76 - RNA, 19 nt, Artificial Sequence
  siRNA
ugaccaggcacuaccgcaa

SEQ ID NO: 77 - RNA, 19 nt, Artificial Sequence
  siRNA
gugcauaaacugaccggaa

SEQ ID NO: 78 - RNA, 19 nt, Artificial Sequence
  siRNA
ccucaaaguuaaggcauaa

SEQ ID NO: 79 - RNA, 19 nt, Artificial Sequence
  siRNA
agaaacgagcugaagcgua

SEQ ID NO: 80 - RNA, 19 nt, Artificial Sequence
  siRNA
cuuaccaggcugcgcgcaa

SEQ ID NO: 81 - RNA, 19 nt, Artificial Sequence
  siRNA
gaauucuccaggcgaaaua

SEQ ID NO: 82 - RNA, 19 nt, Artificial Sequence
  siRNA
gggaaagccaggcgcauuu

SEQ ID NO: 83 - RNA, 19 nt, Artificial Sequence
  siRNA
ccagugauuuggaggcgaa

SEQ ID NO: 84 - RNA, 19 nt, Artificial Sequence
  siRNA
uaacgaugggcuucggaga

SEQ ID NO: 85 - RNA, 19 nt, Artificial Sequence
  siRNA
cgagauaaugacagcgugu

SEQ ID NO: 86 - RNA, 19 nt, Artificial Sequence
  siRNA
cugcaaagguuaucguuca

SEQ ID NO: 87 - RNA, 19 nt, Artificial Sequence
  siRNA
aauacuagagcaaccgaaa

SEQ ID NO: 88 - RNA, 19 nt, Artificial Sequence
  siRNA
cgacgauccuuucggaacu

SEQ ID NO: 89 - RNA, 19 nt, Artificial Sequence
  siRNA
ggguaagauaugaauucga

SEQ ID NO: 90 - RNA, 19 nt, Artificial Sequence
  siRNA
guagagugugucuucgaua

SEQ ID NO: 91 - RNA, 19 nt, Artificial Sequence
  siRNA
gcguacagaaggcacggua

SEQ ID NO: 92 - RNA, 19 nt, Artificial Sequence
  siRNA
auggagaagacucggauga

SEQ ID NO: 93 - RNA, 19 nt, Artificial Sequence
  siRNA
acacaauucgccugcguua

SEQ ID NO: 94 - RNA, 19 nt, Artificial Sequence
  siRNA
guaauauaucuguccgauu

SEQ ID NO: 95 - RNA, 19 nt, Artificial Sequence
  siRNA
ccaaagggcagcauccgaa

SEQ ID NO: 96 - RNA, 19 nt, Artificial Sequence
  siRNA
ggacuuagcccucugccga

SEQ ID NO: 97 - RNA, 19 nt, Artificial Sequence
  siRNA
cgguucggagagucggaua

SEQ ID NO: 98 - RNA, 19 nt, Artificial Sequence
  siRNA
aagaagaaccgaucgcaca

SEQ ID NO: 99 - RNA, 19 nt, Artificial Sequence
  siRNA
uuuccauccucuucgauua

SEQ ID NO: 100 - RNA, 19 nt, Artificial Sequence
  siRNA
uagcugauguccacgguga

SEQ ID NO: 101 - RNA, 19 nt, Artificial Sequence
  siRNA
gaaccguccuaccgggaau

SEQ ID NO: 102 - RNA, 19 nt, Artificial Sequence
  siRNA
gaaugaagcugcugcacga

SEQ ID NO: 103 - RNA, 19 nt, Artificial Sequence
  siRNA
aaagaauacuagaguccga

SEQ ID NO: 104 - RNA, 19 nt, Artificial Sequence
  siRNA
cagauauagaacuucgaaa

SEQ ID NO: 105 - RNA, 19 nt, Artificial Sequence
  siRNA
guucccaguuuacggcgaa

SEQ ID NO: 106 - RNA, 19 nt, Artificial Sequence
  siRNA
cuauaucucacccguguua

SEQ ID NO: 107 - RNA, 19 nt, Artificial Sequence
  siRNA
cuauuuaugugccggaaga

SEQ ID NO: 108 - RNA, 19 nt, Artificial Sequence
  siRNA
ggaacuuacacaucgauga

SEQ ID NO: 109 - RNA, 19 nt, Artificial Sequence
  siRNA
cgggauaagaacugcguua

SEQ ID NO: 110 - RNA, 19 nt, Artificial Sequence
  siRNA
gguaaauacaccacgaauu

SEQ ID NO: 111 - RNA, 19 nt, Artificial Sequence
  siRNA
aggacaagucaucgggcua

SEQ ID NO: 112 - RNA, 19 nt, Artificial Sequence
  siRNA
ccgcagcaucagcgccaaa

SEQ ID NO: 113 - RNA, 19 nt, Artificial Sequence
  siRNA
gggcugacccugaaccgaa

SEQ ID NO: 114 - RNA, 19 nt, Artificial Sequence
  siRNA
guaaggaaugaccggaaca

SEQ ID NO: 115 - RNA, 19 nt, Artificial Sequence
  siRNA
cgacaagucuuccggcuac

SEQ ID NO: 116 - RNA, 19 nt, Artificial Sequence
  siRNA
cugcaaaaguguuucgaag

SEQ ID NO: 117 - RNA, 19 nt, Artificial Sequence
  siRNA
cggaaaaccaagacgcuca

SEQ ID NO: 118 - RNA, 19 nt, Artificial Sequence
  siRNA
gcucuguggucaaguccga

SEQ ID NO: 119 - RNA, 19 nt, Artificial Sequence
  siRNA
augaaggagcacccggauu

SEQ ID NO: 120 - RNA, 19 nt, Artificial Sequence
  siRNA
caguacaacuccaugacca

SEQ ID NO: 121 - RNA, 19 nt, Artificial Sequence
  siRNA
ucaggugucucaucggaaa

SEQ ID NO: 122 - RNA, 19 nt, Artificial Sequence
  siRNA
acucgaaugugcaccauaa

SEQ ID NO: 123 - RNA, 19 nt, Artificial Sequence
  siRNA
gccgagugccuaagugaua

SEQ ID NO: 124 - RNA, 19 nt, Artificial Sequence
  siRNA
ggaauugagccacagagua

SEQ ID NO: 125 - RNA, 19 nt, Artificial Sequence
  siRNA
gcacagccaccaugaguua

SEQ ID NO: 126 - RNA, 19 nt, Artificial Sequence
  siRNA
ggaucgagcuacaccugaa

SEQ ID NO: 127 - RNA, 19 nt, Artificial Sequence
  siRNA
gugaacaccaagugcauua

SEQ ID NO: 128 - RNA, 19 nt, Artificial Sequence
  siRNA
ucacugaucccuccaauuc

SEQ ID NO: 129 - RNA, 19 nt, Artificial Sequence
  siRNA
cggaaggacauucgauuca

SEQ ID NO: 130 - RNA, 19 nt, Artificial Sequence
  siRNA
ggacauuacuggccgguuc

SEQ ID NO: 131 - RNA, 19 nt, Artificial Sequence
  siRNA
gcagguggcuggucggaaa

SEQ ID NO: 132 - RNA, 19 nt, Artificial Sequence
  siRNA
gcgcauccacggagacgua

SEQ ID NO: 133 - RNA, 19 nt, Artificial Sequence
  siRNA
aagaccagcucacguggaa

SEQ ID NO: 134 - RNA, 19 nt, Artificial Sequence
  siRNA
gcgaggaacaggacgauaa

SEQ ID NO: 135 - RNA, 19 nt, Artificial Sequence
  siRNA
aguccauggagaagccgaa

SEQ ID NO: 136 - RNA, 19 nt, Artificial Sequence
  siRNA
cuaacagcuuugcgugcua

SEQ ID NO: 137 - DNA, 21 bp, Artificial Sequence
  primer
gtggagaacctactgccatca

SEQ ID NO: 138 - DNA, 21 bp, Artificial Sequence
  primer
gtggcaaccttgtttaggtca

SEQ ID NO: 139 - DNA, 20 bp, Artificial Sequence
  primer
tcgctatccaagctacccct

SEQ ID NO: 140 - DNA, 20 bp, Artificial Sequence
  primer
ccgaccatgccaaccatact

SEQ ID NO: 141 - DNA, 20 bp, Artificial Sequence
  primer
tggctcaaaccactccatcg

SEQ ID NO: 142 - DNA, 20 bp, Artificial Sequence
  primer
cgtcggaagaagcccttaca

SEQ ID NO: 143 - DNA, 20 bp, Artificial Sequence
  primer
ctctcggcttcgacagctac

SEQ ID NO: 144 - DNA, 20 bp, Artificial Sequence
  primer
tccatctgtagcagacacgg

SEQ ID NO: 145 - DNA, 20 bp, Artificial Sequence
  primer
cgcacttaccagctgacgta

SEQ ID NO: 146 - DNA, 20 bp, Artificial Sequence
  primer
gtacacaggctgaccttgct

SEQ ID NO: 147 - DNA, 20 bp, Artificial Sequence
  primer
gggacacttccatgtccagg

SEQ ID NO: 148 - DNA, 20 bp, Artificial Sequence
  PRIMER
ttcacgtgcattaggtcgct

SEQ ID NO: 149 - DNA, 16 bp, Artificial Sequence
  primer
cctcctccgccagctt

SEQ ID NO: 150 - DNA, 24 bp, Artificial Sequence
  primer
gtcataacctggttcatcatcact

SEQ ID NO: 151 - DNA, 20 bp, Artificial Sequence
  primer
ggagcaccaacggacctatc

SEQ ID NO: 152 - DNA, 20 bp, Artificial Sequence
  primer
cagggccttctggatgagtg

SEQ ID NO: 153 - DNA, 20 bp, Artificial Sequence
  primer
caggcagcccagactagatt

SEQ ID NO: 154 - DNA, 20 bp, Artificial Sequence
  primer
tattggagtcttcggggcca

SEQ ID NO: 155 - DNA, 20 bp, Artificial Sequence
  primer
cctatgctgggtggactctc

SEQ ID NO: 156 - DNA, 20 bp, Artificial Sequence
  primer
agcaaggcttgtagatgcgg

SEQ ID NO: 157 - DNA, 20 bp, Artificial Sequence
  primer
atgccatacctcaaacggga

SEQ ID NO: 158 - DNA, 21 bp, Artificial Sequence
  primer
ccgtttctcttgatggcacct

SEQ ID NO: 159 - DNA, 20 bp, Artificial Sequence
  primer
ggcaagatggagggctcttt

SEQ ID NO: 160 - DNA, 20 bp, Artificial Sequence
  primer
cgcagagtaatgtgtgctgc

SEQ ID NO: 161 - DNA, 20 bp, Artificial Sequence
  primer
tatccaggctggtctgcaag

SEQ ID NO: 162 - DNA, 20 bp, Artificial Sequence
  primer
gcagctgtcattcttggacc

SEQ ID NO: 163 - DNA, 21 bp, Artificial Sequence
  primer
cctggcgtcgtgattagtgat

SEQ ID NO: 164 - DNA, 22 bp, Artificial Sequence
  primer
agacgttcagtcctgtccataa

SEQ ID NO: 165 - RNA, 19 nt, Artificial Sequence
  siRNA
caacggaccuaucgauguc

SEQ ID NO: 166 - RNA, 19 nt, Artificial Sequence
  siRNA
uagcauaugugaccuauca

SEQ ID NO: 167 - RNA, 19 nt, Artificial Sequence
  siRNA
guaagcaacugauggcauu

SEQ ID NO: 168 - RNA, 19 nt, Artificial Sequence
  siRNA
gaacagaucgucauugcag

SEQ ID NO: 169 - RNA, 19 nt, Artificial Sequence
  siRNA
gcacacaucgugagacguu

SEQ ID NO: 170 - RNA, 19 nt, Artificial Sequence
  siRNA
ugacuaaccugccgcuuug

SEQ ID NO: 171 - RNA, 19 nt, Artificial Sequence
  siRNA
caaggacgaugcauuuaca

SEQ ID NO: 172 - RNA, 19 nt, Artificial Sequence
  siRNA
ggacuauuccgacccauug

SEQ ID NO: 173 - RNA, 19 nt, Artificial Sequence
  siRNA
gauauucucuuugcuaugc

SEQ ID NO: 174 - RNA, 19 nt, Artificial Sequence
  siRNA
guaagugaguucaucaguu

SEQ ID NO: 175 - RNA, 19 nt, Artificial Sequence
  siRNA
gaaugugucaggugcauaa

SEQ ID NO: 176 - RNA, 18 nt, Artificial Sequence
  siRNA
uaugcaagcuccauguua

SEQ ID NO: 177 - RNA, 19 nt, Artificial Sequence
  siRNA
gcaaauacacuacgaacaa

SEQ ID NO: 178 - RNA, 19 nt, Artificial Sequence
  siRNA
ccaaggagucugugagaaa

SEQ ID NO: 179 - RNA, 19 nt, Artificial Sequence
  siRNA
gagcagcaguucugaagag

SEQ ID NO: 180 - RNA, 19 nt, Artificial Sequence
  siRNA
gaacaacgugucucucugc

SEQ ID NO: 181 - RNA, 19 nt, Artificial Sequence
  siRNA
cagcgaauguuuccuaaau

SEQ ID NO: 182 - RNA, 19 nt, Artificial Sequence
  siRNA
cgagacaaaucccgggaaa

SEQ ID NO: 183 - RNA, 19 nt, Artificial Sequence
  siRNA
acacuuaccagccgacgua

SEQ ID NO: 184 - RNA, 19 nt, Artificial Sequence
  siRNA
gaugucggcucacuccaua

SEQ ID NO: 185 - RNA, 19 nt, Artificial Sequence
  siRNA
gcaagagacaauuauggua

SEQ ID NO: 186 - RNA, 19 nt, Artificial Sequence
  siRNA
ugccaaauaugaauaacga

SEQ ID NO: 187 - RNA, 19 nt, Artificial Sequence
  siRNA
cgauuuagcugacaucaag

SEQ ID NO: 188 - RNA, 19 nt, Artificial Sequence
  siRNA
cgucacacaucccaucaga